European Patent Application EP 4 269 592 A1, published November 1, 2023. Title: Novel DNA polymerase. Applicant: NIPPON GENE CO., LTD. The sequence listing filed with the application follows.

SEQUENCE LISTING (30 sequences)

SEQ ID NO: 1 - DNA, 5741 bp, Artificial sequence
  vector
ttctcatgtttgacagcttatcatcgataagctttaatgcggtagtttatcacagttaaattgctaacgcagtcaggcaccgtgtatgaaatctaacaatgcgctcatcgtcatcctcggcaccgtcaccctggatgctgtaggcataggcttggttatgccggtactgccgggcctcttgcgggatatccggatatagttcctcctttcagcaaaaaacccctcaagacccgtttagaggccccaaggggttatgctagttattgctcagcggtggcagcagccaactcagcttcctttcgggctttgttagcagccggatcctcgagcataccggtatggagctcgtcgacctgctgatgcatatggctgccgcgcggcaccaggccgctgctgtgatgatgatgatgatggctgctgcccatggtatatctccttcttaaagttaaacaaaattatttctagaggggaattgttatccgctcacaattcccctatagtgagtcgtattaatttcgcgggatcgagatctcgatcctctacgccggacgcatcgtggccggcatcaccggcgccacaggtgcggttgctggcgcctatatcgccgacatcaccgatggggaagatcgggctcgccacttcgggctcatgagcgcttgtttcggcgtgggtatggtggcaggccccgtggccgggggactgttgggcgccatctccttgcatgcaccattccttgcggcggcggtgctcaacggcctcaacctactactgggctgcttcctaatgcaggagtcgcataagggagagcgtcgagatcccggacaccatcgaatggcgcaaaacctttcgcggtatggcatgatagcgcccggaagagagtcaattcagggtggtgaatgtgaaaccagtaacgttatacgatgtcgcagagtatgccggtgtctcttatcagaccgtttcccgcgtggtgaaccaggccagccacgtttctgcgaaaacgcgggaaaaagtggaagcggcgatggcggagctgaattacattcccaaccgcgtggcacaacaactggcgggcaaacagtcgttgctgattggcgttgccacctccagtctggccctgcacgcgccgtcgcaaattgtcgcggcgattaaatctcgcgccgatcaactgggtgccagcgtggtggtgtcgatggtagaacgaagcggcgtcgaagcctgtaaagcggcggtgcacaatcttctcgcgcaacgcgtcagtgggctgatcattaactatccgctggatgaccaggatgccattgctgtggaagctgcctgcactaatgttccggcgttatttcttgatgtctctgaccagacacccatcaacagtattattttctcccatgaagacggtacgcgactgggcgtggagcatctggtcgcattgggtcaccagcaaatcgcgctgttagcgggcccattaagttctgtctcggcgcgtctgcgtctggctggctggcataaatatctcactcgcaatcaaattcagccgatagcggaacgggaaggcgactggagtgccatgtccggttttcaacaaaccatgcaaatgctgaatgagggcatcgttcccactgcgatgctggttgccaacgatcagatggcgctgggcgcaatgcgcgccattaccgagtccgggctgcgcgttggtgcggatatctcggtagtgggatacgacgataccgaagacagctcatgttatatcccgccgttaaccaccatcaaacaggattttcgcctgctggggcaaaccagcgtggaccgcttgctgcaactctctcagggccaggcggtgaagggcaatcagctgttgcccgtctcactggtgaaaagaaaaaccaccctggcgcccaatacgcaaaccgcctctccccgcgcgttggccgattcattaatgcagctggcacgacaggtttcccgactggaaagcgggcagtgagcgcaacgcaattaatgtaagttagctcactcattaggcaccgggatctcgaccgatgcccttgagagccttcaacccagtcagctccttccggtgggcgcggggcatgactatcgtcgccgcacttatgactgtcttctttatcatgcaactcgtaggacaggtgccggcagcgctctgggtcattttcggcgaggaccgctttcgctggagcgcgacgatgatcggcctgtcgcttgcggtattcggaatcttgcacgccctcgctcaagccttcgtcactggtcccgccaccaaacgtttcggcgagaagcaggccattatcgccggcatggcggccgacgcgctgggctacgtcttgctggcgttcgcgacgcgaggctggatggccttccccattatgattcttctcgcttccggcggcatcgggatgcccgcgttgcaggccatgctgtccaggcaggtagatgacgaccatcagggacagcttcaaggatcgctcgcggctcttaccagcctaacttcgatcactggaccgctgatcgtcacggcgatttatgccgcctcggcgagcacatggaacgggttggcatggattgtaggcgccgccctataccttgtctgcctccccgcgttgcgtcgcggtgcatggagccgggccacctcgacctgaatggaagccggcggcacctcgctaacggattcaccactccaagaattggagccaatcaattcttgcggagaactgtgaatgcgcaaaccaacccttggcagaacatatccatcgcgtccgccatctccagcagccgcacgcggcgcatctcgggcagcgttgggtcctggccacgggtgcgcatgatcgtgctcctgtcgttgaggacccggctaggctggcggggttgccttactggttagcagaatgaatcaccgatacgcgagcgaacgtgaagcgactgctgctgcaaaacgtctgcgacctgagcaacaacatgaatggtcttcggtttccgtgtttcgtaaagtctggaaacgcggaagtcagcgccctgcaccattatgttccggatctgcatcgcaggatgctgctggctaccctgtggaacacctacatctgtattaacgaagcgctggcattgaccctgagtgatttttctctggtcccgccgcatccataccgccagttgtttaccctcacaacgttccagtaaccgggcatgttcatcatcagtaacccgtatcgtgagcatcctctctcgtttcatcggtatcattacccccatgaacagaaatcccccttacacggaggcatcagtgaccaaacaggaaaaaaccgcccttaacatggcccgctttatcagaagccagacattaacgcttctggagaaactcaacgagctggacgcggatgaacaggcagacatctgtgaatcgcttcacgaccacgctgatgagctttaccgcagctgcctcgcgcgtttcggtgatgacggtgaaaacctctgacacatgcagctcccggagacggtcacagcttgtctgtaagcggatgccgggagcagacaagcccgtcagggcgcgtcagcgggtgttggcgggtgtcggggcgcagccatgacccagtcacgtagcgatagcggagtgtatactggcttaactatgcggcatcagagcagattgtactgagagtgcaccatatatgcggtgtgaaataccgcacagatgcgtaaggagaaaataccgcatcaggcgctcttccgcttcctcgctcactgactcgctgcgctcggtcgttcggctgcggcgagcggtatcagctcactcaaaggcggtaatacggttatccacagaatcaggggataacgcaggaaagaacatgtgagcaaaaggccagcaaaaggccaggaaccgtaaaaaggccgcgttgctggcgtttttccataggctccgcccccctgacgagcatcacaaaaatcgacgctcaagtcagaggtggcgaaacccgacaggactataaagataccaggcgtttccccctggaagctccctcgtgcgctctcctgttccgaccctgccgcttaccggatacctgtccgcctttctcccttcgggaagcgtggcgctttctcatagctcacgctgtaggtatctcagttcggtgtaggtcgttcgctccaagctgggctgtgtgcacgaaccccccgttcagcccgaccgctgcgccttatccggtaactatcgtcttgagtccaacccggtaagacacgacttatcgccactggcagcagccactggtaacaggattagcagagcgaggtatgtaggcggtgctacagagttcttgaagtggtggcctaactacggctacactagaaggacagtatttggtatctgcgctctgctgaagccagttaccttcggaaaaagagttggtagctcttgatccggcaaacaaaccaccgctggtagcggtggtttttttgtttgcaagcagcagattacgcgcagaaaaaaaggatctcaagaagatcctttgatcttttctacggggtctgacgctcagtggaacgaaaactcacgttaagggattttggtcatgagattatcaaaaaggatcttcacctagatccttttaaattaaaaatgaagttttaaatcaatctaaagtatatatgagtaaacttggtctgacagttaccaatgcttaatcagtgaggcacctatctcagcgatctgtctatttcgttcatccatagttgcctgactccccgtcgtgtagataactacgatacgggagggcttaccatctggccccagtgctgcaatgataccgcgagacccacgctcaccggctccagatttatcagcaataaaccagccagccggaagggccgagcgcagaagtggtcctgcaactttatccgcctccatccagtctattaattgttgccgggaagctagagtaagtagttcgccagttaatagtttgcgcaacgttgttgccattgctgcaggcatcgtggtgtcacgctcgtcgtttggtatggcttcattcagctccggttcccaacgatcaaggcgagttacatgatcccccatgttgtgcaaaaaagcggttagctccttcggtcctccgatcgttgtcagaagtaagttggccgcagtgttatcactcatggttatggcagcactgcataattctcttactgtcatgccatccgtaagatgcttttctgtgactggtgagtactcaaccaagtcattctgagaatagtgtatgcggcgaccgagttgctcttgcccggcgtcaacacgggataataccgcgccacatagcagaactttaaaagtgctcatcattggaaaacgttcttcggggcgaaaactctcaaggatcttaccgctgttgagatccagttcgatgtaacccactcgtgcacccaactgatcttcagcatcttttactttcaccagcgtttctgggtgagcaaaaacaggaaggcaaaatgccgcaaaaaagggaataagggcgacacggaaatgttgaatactcatactcttcctttttcaatattattgaagcatttatcagggttattgtctcatgagcggatacatatttgaatgtatttagaaaaataaacaaataggggttccgcgcacatttccccgaaaagtgccacctgacgtctaagaaaccattattatcatgacattaacctataaaaataggcgtatcacgaggccctttcgtcttcaagaa

SEQ ID NO: 2 - DNA, 25 bp, Artificial sequence
  Primer
gggcatatggaggcgatgcttccgc

SEQ ID NO: 3 - DNA, 29 bp, Artificial sequence
  Primer
ggggtcgacctaacccttggcggaaagcc

SEQ ID NO: 4 - DNA, 2505 bp, Thermus thermophilus
atggaggcgatgcttccgctctttgaatccaaaggccgggtcctcctggtggacggccaccacctggcctaccgcaccttcttcgccctgaagggcctcaccacgagccggggcgaaccggtgcaggcggtctacggcttcgccaagagcctcctcaaggccctgaaggaggacgggtacaagtccgtcttcgtggtctttgacgccaaggccccctccttccgccacgaggcctacgaggcctacaaggcggggagggccccgacccccgaggacttcccccggcagctcgccctcatcaaggagctggtggacctcctggggtttactcgcctcgaggtccccggctacgaggcggacgacgtcctcgccaccctggccaagaaggcggaaaaggaggggtacgaggtgcgcatcctcaccgccgaccgggacctctaccagctcgtctccgaccgcgtcgccgtcctccaccccgagggccacctcatcaccccggagtggctttgggagaagtacggcctcaggccggagcagtgggtggacttccgcgccctcgtgggggacccctccgacaacctccccggggtcaagggcatcggggagaagaccgccctcaagctcctcaaggagtggggaagcctggaaagcctcctcaagaacctggaccgggtgaagccggaaaacgtccgggagaagatcaaggcccacctggaagacctcaggctctccttggagctctcccgggtgcgcgccgacctccccctggaggtggacctcgcccaggggcgggagcccgaccgggaggggcttagggccttcctggagaggctggagttcggcagcctcctccacgagttcggcctcctggaggcccccacccccctggaggaggccccctggcccccgccggaaggggccttcgtgggcttcgtcctctcccgccccgagcccatgtgggcggagcttaaagccctggccgcctgcagggacggccgggtgcaccgggcagaggaccccttggcgggacttggggacctcgaggaggtccggggcctcctcgccaaggacctcgccgtcttggccttgagggaggggctggatctggccccaggggacgaccccatgctcctcgcctacctcctggacccctccaacaccacccccgagggggtggcgcggcgctacgggggggagtggacggaagacgccgcccaccgggccctcctctcggagaggctccatcggaacctccttaagcgcctcgagggggaggagaagctcctttggctctaccacgaggtggaaaagcccctctcccgggtcctggcccacatggaggccaccggggtacggctggacgtggcctacttgcaggccctttccctggagcttgcggaggagatccgccgcctcgaggaggaggtcttccgcttggcgggccaccccttcaacctcaactcccgggaccagctggaaagggtgctctttgacgagcttaggcttcccgccttggggaagacgcaaaagacgggcaagcgctccaccagcgccgcggtgctggaggccctacgggaggcccaccccatcgtggagaagatcctccagcaccgggagctcaccaagctcaagaacacctacgtggaccccctcccaagcctcgtccacccgaggacgggccgcctccacacccgcttcaaccagacggccacggccacggggaggcttagtagctccgaccccaacctgcagaacatccccgtccgcacccccttgggccagaggatccgccgggccttcgtggccgaggcgggttgggcgttggtggccctggactatagccagatagagctccgcgtcctcgcccacctctccggggacgaaaacctgatcagggtcttccaggaggggaaggacatccacacccagaccgcaagctggatgttcggcgtccccccggaggccgtggaccccctgatgcgccgggcggccaagacggtgaacttcggcgtcctctacggcatgtccgcccataggctctcccaggagcttgccatcccctacgaggaggcggtggcctttatagagcgctacttccaaagcttccccaaggtgcgggcctggatagaaaagaccctggaggaggggaggaagcggggctacgtggaaaccctcttcggaagaaggcgctacgtgcccgacctcaacgcccgggtgaagagcgtcagggaggccgcggagcgcatggccttcaacatgcccgtccagggcaccgccgccgacctcatgaagctcgccatggtgaagctcttcccccgcctccgggagatgggggcccgcatgctcctccaggtccacgacgagctcctcctggaggccccccaagcgcgggccgaggaggtggcggctttggccaaggaggccatggagaaggcctatcccctcgccgtgcccctggaggtggaggtggggatcggggaggactggctttccgccaagggttag

SEQ ID NO: 5 - protein, 834 aa, Thermus thermophilus
MEAMLPLFESKGRVLLVDGHHLAYRTFFALKGLTTSRGEPVQAVYGFAKSLLKALKEDGYKSVFVVFDAKAPSFRHEAYEAYKAGRAPTPEDFPRQLALIKELVDLLGFTRLEVPGYEADDVLATLAKKAEKEGYEVRILTADRDLYQLVSDRVAVLHPEGHLITPEWLWEKYGLRPEQWVDFRALVGDPSDNLPGVKGIGEKTALKLLKEWGSLESLLKNLDRVKPENVREKIKAHLEDLRLSLELSRVRADLPLEVDLAQGREPDREGLRAFLERLEFGSLLHEFGLLEAPTPLEEAPWPPPEGAFVGFVLSRPEPMWAELKALAACRDGRVHRAEDPLAGLGDLEEVRGLLAKDLAVLALREGLDLAPGDDPMLLAYLLDPSNTTPEGVARRYGGEWTEDAAHRALLSERLHRNLLKRLEGEEKLLWLYHEVEKPLSRVLAHMEATGVRLDVAYLQALSLELAEEIRRLEEEVFRLAGHPFNLNSRDQLERVLFDELRLPALGKTQKTGKRSTSAAVLEALREAHPIVEKILQHRELTKLKNTYVDPLPSLVHPRTGRLHTRFNQTATATGRLSSSDPNLQNIPVRTPLGQRIRRAFVAEAGWALVALDYSQIELRVLAHLSGDENLIRVFQEGKDIHTQTASWMFGVPPEAVDPLMRRAAKTVNFGVLYGMSAHRLSQELAIPYEEAVAFIERYFQSFPKVRAWIEKTLEEGRKRGYVETLFGRRRYVPDLNARVKSVREAAERMAFNMPVQGTAADLMKLAMVKLFPRLREMGARMLLQVHDELLLEAPQARAEEVAALAKEAMEKAYPLAVPLEVEVGIGEDWLSAKG

SEQ ID NO: 6 - DNA, 31 bp, Artificial sequence
  Primer
gaagagcgtcagggagcgcgcggagcgcatg

SEQ ID NO: 7 - DNA, 31 bp, Artificial sequence
  Primer
catgcgctccgcgcgctccctgacgctcttc

SEQ ID NO: 8 - DNA, 31 bp, Artificial sequence
  Primer
gaagagcgtcaggcgcgccgcggagcgcatg

SEQ ID NO: 9 - DNA, 31 bp, Artificial sequence
  Primer
catgcgctccgcggcgcgcctgacgctcttc

SEQ ID NO: 10 - DNA, 31 bp, Artificial sequence
  Primer
gaagagcgtccgtcgccgcgcggagcgcatg

SEQ ID NO: 11 - DNA, 31 bp, Artificial sequence
  Primer
catgcgctccgcgcggcgacggacgctcttc

SEQ ID NO: 12 - DNA, 31 bp, Artificial sequence
  Primer
gaagagcgtccgtaagaaagcggagcgcatg

SEQ ID NO: 13 - DNA, 31 bp, Artificial sequence
  Primer
catgcgctccgctttcttacggacgctcttc

SEQ ID NO: 14 - DNA, 26 bp, Artificial sequence
  Primer
gtgttttatctctgcgagcataatgc

SEQ ID NO: 15 - DNA, 25 bp, Artificial sequence
  Primer
catccacacgcagcagcgtctgttc

SEQ ID NO: 16 - DNA, 23 bp, Artificial sequence
  Primer
atgacgatatcgctgcgctggtc

SEQ ID NO: 17 - DNA, 22 bp, Artificial sequence
  Primer
ctggccgtcaggcagctcatag

SEQ ID NO: 18 - DNA, 20 bp, Artificial sequence
  Primer
aaattttggggaccaggaac

SEQ ID NO: 19 - DNA, 20 bp, Artificial sequence
  Primer
tggcagctgtgtaggtcaac

SEQ ID NO: 20 - DNA, 20 bp, Artificial sequence
  Primer
atgtcgcgcattggcatgga

SEQ ID NO: 21 - DNA, 3665 bp, Artificial sequence
  Plasmid
gttttcccagtcacgacgttgtaaaacgacggccagtgaattgtaatagctctctgagtacggaacactctttcccttaacgacgctcttccgatctgatctaatacgactcactatagggagaccaaaagatcacattggcacccgcaatcctgctaacaatgctgcaatcgtgctacaacttcctcaaggaacaacattgccaaaaggcttctacgcagaagggagcagaggcggcagtcaagcctcttctcgttcctcatcacgtagtcgcaacagttcaagaaattcaactccaggcagcagtaggggaacttctcctgctagaatggctggcaatggcggtgatgctgctcttgctttgctgctgcttgacagattgaaccagcttgagagcaaaatgtctggtaaaggccaacaacaacaaggccaaactgtcactaagaaatctgctgctgaggcttctaagaagcctcggcaaaaacgtactgccactaaagcatacaatgtaacacaagctttcggcagacgtggtccagaacaaacccaaggaaattttggggaccaggaactaatcagacaaggaactgattacaaacattggccgcaaattgcacaatttgcccccagcgcttcagcgttcttcggaatgtcgcgcattggcatggaagtcacaccttcgggaacgtggttgacctacacaggtgccatcaaattggatgacaaagatccaaatttcaaagatcaagtcattttgctgaataagcatattgacctcttctatagtgtcacctaaatgatcagatcggaagagcacacgtctgaactccagtcttcaatggtatcgcccagatagcttggcgtaatcatggtcatggtcatagctgtttcctgtgtgaaattgttatccgctcacaattccacacaacatacgagccggaagcataaagtgtaaagcctggggtgcctaatgagtgagctaactcacattaattgcgttgcgctcactgcccgctttccagtcgggaaacctgtcgtgccagctgcattaatgaatcggccaacgcgcggggagaggcggtttgcgtattgggcgctcttccgcttcctcgctcactgactcgctgcgctcggtcgttcggctgcggcgagcggtatcagctcactcaaaggcggtaatacggttatccacagaatcaggggataacgcaggaaagaacatgtgagcaaaaggccagcaaaaggccaggaaccgtaaaaaggccgcgttgctggcgtttttccataggctccgcccccctgacgagcatcacaaaaatcgacgctcaagtcagaggtggcgaaacccgacaggactataaagataccaggcgtttccccctggaagctccctcgtgcgctctcctgttccgaccctgccgcttaccggatacctgtccgcctttctcccttcgggaagcgtggcgctttctcatagctcacgctgtaggtatctcagttcggtgtaggtcgttcgctccaagctgggctgtgtgcacgaaccccccgttcagcccgaccgctgcgccttatccggtaactatcgtcttgagtccaacccggtaagacacgacttatcgccactggcagcagccactggtaacaggattagcagagcgaggtatgtaggcggtgctacagagttcttgaagtggtggcctaactacggctacactagaagaacagtatttggtatctgcgctctgctgaagccagttaccttcggaaaaagagttggtagctcttgatccggcaaacaaaccaccgctggtagcggtggtttttttgtttgcaagcagcagattacgcgcagaaaaaaaggatctcaagaagatcctttgatcttttctacggggtctgacgctcagtggaacgaaaactcacgttaagggattttggtcatgagattatcaaaaaggatcttcacctagatccttttaaattaaaaatgaagttttaaatcaatctaaagtatatatgagtaaacttggtctgacagttaccaatgcttaatcagtgaggcacctatctcagcgatctgtctatttcgttcatccatagttgcctgactccccgtcgtgtagataactacgatacgggagggcttaccatctggccccagtgctgcaatgataccgcgagacccacgctcaccggctccagatttatcagcaataaaccagccagccggaagggccgagcgcagaagtggtcctgcaactttatccgcctccatccagtctattaattgttgccgggaagctagagtaagtagttcgccagttaatagtttgcgcaacgttgttgccattgctacaggcatcgtggtgtcacgctcgtcgtttggtatggcttcattcagctccggttcccaacgatcaaggcgagttacatgatcccccatgttgtgcaaaaaagcggttagctccttcggtcctccgatcgttgtcagaagtaagttggccgcagtgttatcactcatggttatggcagcactgcataattctcttactgtcatgccatccgtaagatgcttttctgtgactggtgagtactcaaccaagtcattctgagaatagtgtatgcggcgaccgagttgctcttgcccggcgtcaatacgggataataccgcgccacatagcagaactttaaaagtgctcatcattggaaaacgttcttcggggcgaaaactctcaaggatcttaccgctgttgagatccagttcgatgtaacccactcgtgcacccaactgatcttcagcatcttttactttcaccagcgtttctgggtgagcaaaaacaggaaggcaaaatgccgcaaaaaagggaataagggcgacacggaaatgttgaatactcatactcttcctttttcaatattattgaagcatttatcagggttattgtctcatgagcggatacatatttgaatgtatttagaaaaataaacaaataggggttccgcgcacatttccccgaaaagtgccacctgacgtctaagaaaccattattatcatgacattaacctataaaaataggcgtatcacgaggccctttcgtctcgcgcgtttcggtgatgacggtgaaaacctctgacacatgcagctcccggagacggtcacagcttgtctgtaagcggatgccgggagcagacaagcccgtcagggcgcgtcagcgggtgttggcgggtgtcggggctggcttaattaaatgccccaaaacatcaggttaatggcgttcttgatgtcattctcgcgatgcgacagatccgcaacctcttcgccaattaccgacactggtactgacgccatatccgtggtcatcatacgccagctttcatccccaatgtggacaaccggatagagttcacgggaaactttgtcgctcagtaaccgtgcagaagccaacggaatcaccgtgcgacgaccaggagtatcgatgatgtcgctttgcacatccacaaacaggcgatagcgactttcgcgtttgtaggtgtagactttgaactgcggtacgttacagagagcgcaactgctgtgacggacgatctgtacgcgcttcttcgctattccgccaactcgcaaacggaggatgtgctgcaaggcgattaagttgggtaacgcctgg

SEQ ID NO: 22 - RNA, 741 nt, Artificial sequence
  Control RNA
gggagaccaaaagaucacauuggcacccgcaauccugcuaacaaugcugcaaucgugcuacaacuuccucaaggaacaacauugccaaaaggcuucuacgcagaagggagcagaggcggcagucaagccucuucucguuccucaucacguagucgcaacaguucaagaaauucaacuccaggcagcaguaggggaacuucuccugcuagaauggcuggcaauggcggugaugcugcucuugcuuugcugcugcuugacagauugaaccagcuugagagcaaaaugucugguaaaggccaacaacaacaaggccaaacugucacuaagaaaucugcugcugaggcuucuaagaagccucggcaaaaacguacugccacuaaagcauacaauguaacacaagcuuucggcagacgugguccagaacaaacccaaggaaauuuuggggaccaggaacuaaucagacaaggaacugauuacaaacauuggccgcaaauugcacaauuugcccccagcgcuucagcguucuucggaaugucgcgcauuggcauggaagucacaccuucgggaacgugguugaccuacacaggugccaucaaauuggaugacaaagauccaaauuucaaagaucaagucauuuugcugaauaagcauauugaccucuucuauagugucaccuaaaugaucagaucggaagagcacacgucugaacuccagucuucaaugguaucgcccagauagcuu

SEQ ID NO: 23 - DNA, 25 bp, Artificial sequence
  Primer
tcacccacactgtgcccatctacga

SEQ ID NO: 24 - DNA, 25 bp, Artificial sequence
  Primer
cagcggaaccgctcattgccaatgg

SEQ ID NO: 25 - DNA, 25 bp, Artificial sequence
  Primer
aaacttgccatcccctacgaggagg

SEQ ID NO: 26 - DNA, 25 bp, Artificial sequence
  Primer
ctgcttgccatcccctacgaggagg

SEQ ID NO: 27 - DNA, 25 bp, Artificial sequence
  Primer
tatcttgccatcccctacgaggagg

SEQ ID NO: 28 - DNA, 22 bp, Artificial sequence
  Primer
ctgggagagcctatgggcggac

SEQ ID NO: 29 - DNA, 20 bp, Artificial sequence
  Primer
ttacaaacattggccgcaaa

SEQ ID NO: 30 - DNA, 18 bp, Artificial sequence
  Primer
gcgcgacattccgaagaa